European Patent Specification EP 4 522 990 B1, published March 25, 2026. Title: USE FO BMMF1 REP PROTEIN AS DIAGNOSTIC MARKER FOR PANCREATIC CANCER AND DIABETES MELLITUS TYPE 2. Applicant: Deutsches Krebsforschungszentrum Stiftung des Oeffentlichen Rechts. Application EP, filed May 11, 2023. The sequence listing filed with the application follows.

SEQUENCE LISTING (24 sequences)

SEQ ID NO: 1 - protein, 324 aa, Homo sapiens
MSDLIVKDNALMNASYNLALVEQRLILLAIIEARETGKGINANDPLTVHASSYINQFNVERHTAYQALKDACKDLFARQFSYQEKRERGRINITSRWVSQIGYMDDTATVEIIFAPAVVPLITRLEEQFTQYDIEQISGLSSAYAVRMYELLICWRSTGKTPIIELDEFRKRIGVLDTEYTRTDNLKMRVIELALKQINEHTDITASYEQHKKGRVITGFSFKFKHKKQNSDKTPKNSDSSPRIVKHSQIPTNIVKQPENAKMSDLEHRASRVTGEIMRNRLSDRFKQGDESAIDMMKRIQSEIITDAIADQWESKLEEFGVVF

SEQ ID NO: 2 - protein, 18 aa, Homo sapiens
EARETGKGINANDPLTVH

SEQ ID NO: 3 - protein, 21 aa, Homo sapiens
KQINEHTDITASYEQHKKGRT

SEQ ID NO: 4 - protein, 8 aa, synthetic construct
GAHHHHHH

SEQ ID NO: 5 - protein, 11 aa, synthetic construct
MASMTGGQQMG

SEQ ID NO: 6 - protein, 8 aa, synthetic construct
DYKDDDDK

SEQ ID NO: 7 - protein, 8 aa, synthetic construct
WSHPQFEK

SEQ ID NO: 8 - protein, 319 aa, Homo sapiens
MSKLVVKDNALMNASYNLDLVEQRLILLAIIEARESGKGINANDPLTVHAESYINQFGVHRVTAYQALKDACDNLFARQFSYQSKSEKGNIQNHRSRWVSEIIYIDTEATVKIIFAPAIVPLITRLEEQFTKYDIEQISDLSSAYAIRLYELLICWRSTGKTPIIGLGEFRNRVGVLDSEYHRIAHLKERVIEHSIKQINEHTDITATYEQHKKGRTITGFSFKFKQKKPKQAEIATETPKTATNDPDTTKPLTEPQIAKYSMILCKLGSISDLSNFPDYPAFANWIGNILRNPEKADEQIAKRIFTALKTETDYSKKN

SEQ ID NO: 9 - protein, 7 aa, Homo sapiens
NRLSDRF

SEQ ID NO: 10 - protein, 326 aa, unidentified
MSDLIVKDNALMNASYNLALVEQRLILLAILEARETGKGINANDPLTVHASSYINQFNVERHTAYQALKDACKDLFARQFSYQEKRERGRINITSRWVSQIGYMDDTATVEIIFAPAVVPLITRLEEQFTQYDIEQISELSSAYAVRLYELLICWRSTGKTPIIDLTEFRKRLGVLDTEYTRTDNLKMRVIELGLKQINEHTDITASYEQHKKGRTITGFSFKFKQKKKTGAEMPKNSDSSPHIEKPSQIPANIAKQPENAKKDDLGHRASKITGLIMSNGLADRFKRGDESVIDMMKRIKEEITTDTTADQWENKLEEFGVIFQS

SEQ ID NO: 11 - protein, 324 aa, unidentified
MSDLIVKDNALMNASYNLDLVEQRLILLAILEARETGKGINANDPLTVHAESYINQFGVARQTAYQALKDACKDLFARQFSYQEKRERGRANITSRWVSQIAYIDETATVEVIFAPAVVPLITRLEEQFTQYDIEQISGLSSAYAVRLYELLICWRSTGKTPVIELAEFRKRLGVLNDEYTRSDNFKKWIIENPIKQINEHTDITASYEQHKKGRTITGFSFKFKQKKKTEPETPKNSDSSQRIEKPSQIPANIVKQPENANLSDLQHRASKITGLIMSNRLSDRFKQGDESIMQMMARIQSEITTDSIADQWQSKLEEFGVVF

SEQ ID NO: 12 - protein, 324 aa, unidentified
MSDLIVKDNALMNASYNLALVEQRLILLAILEARETGKGINANDPLTVHASSYINQFNVERHTAYQALKDACKDLFARQFSYQEKRERGRANITSRWVSQIAYIDETATVEVIFAPAVVPLITRLEEQFTQYDIEQISGLSSAYAVRLYELLICWRTTGKTPVLDLTEFRKRLGVLDTEYTRTDNLKMRVIEQSLKQINKHTDITASYEQHKKGRTITGFSFKFKQKKKTEPETPKNNDSGVSKPKTVEIPAEVVKQPKNTNLSDLEKRVRMITGAIAKNNLASRFQHGNESPLDMMKRIQSEITSDETADLWQNKLESMGVVF

SEQ ID NO: 13 - DNA, 999 bp, unidentified
  source 1..999: mol_type = other DNA
atgagcgacctgatcgtgaaagacaatgccctgatgaacgcctcctacaacctggcactggtcgaacagagactgattctgctggctatcatcgaggcaagggagaccggcaagggcatcaacgccaatgaccccctgacagtgcacgccagctcctacatcaaccagtttaatgtggagcgccacaccgcctatcaggccctgaaggacgcctgcaaggatctgtttgcccggcagttcagctaccaggagaagcgggagagaggcaggatcaacatcacaagcagatgggtgtcccagatcggctatatggacgataccgccacagtggagatcatctttgcaccagcagtggtgcctctgatcaccaggctggaggagcagttcacacagtacgacatcgagcagatctccggactgtctagcgcctacgccgtgcgcatgtatgagctgctgatctgttggcggtctaccggcaagacacctatcatcgagctggatgagttccgcaagcggatcggcgtgctggacaccgagtacaccagaacagataacctgaagatgagagtgatcgagctggccctgaagcagatcaatgagcacaccgatatcacagcctcttatgagcagcacaagaagggccgcgtgatcaccggcttcagctttaagttcaagcacaagaagcagaactctgacaagacaccaaagaatagcgattcctctccccggatcgtgaagcacagccagatccctaccaacatcgtgaagcagccagagaatgccaagatgtccgacctggagcacagggcatctagggtgacaggcgagatcatgagaaataggctgagcgatcggttcaagcagggcgacgagtccgccatcgatatgatgaagagaatccagtccgagatcatcaccgacgccatcgccgatcagtgggaatctaaactggaagagtttggagtcgtgtttggagcacatcaccatcatcatcactga

SEQ ID NO: 14 - protein, 326 aa, Homo sapiens
MSDLIVKDNALMNASYNLALVEQRLILLAIIEARETGKGINANDPLTVHASSYINQFNVERHTAYQALKDACKDLFARQFSYQEKRERGRINITSRWVSQIGYMDDTATVEIIFAPAVVPLITRLEEQFTQYDIEQISGLSSAYAVRMYELLICWRSTGKTPIIELDEFRKRIGVLDTEYTRTDNLKMRVIELALKQINEHTDITASYEQHKKGRVITGFSFKFKHKKQNSDKTPKNSDSSPRIVKHSQIPTNIVKQPENAKMSDLEHRASRVTGEIMRNRLSDRFKQGDESAIDMMKRIQSEIITDAIADQWESKLEEFGVVFGA

SEQ ID NO: 15 - DNA, 974 bp, Homo sapiens
  source 1..974: mol_type = genomic DNA
atgagcgatttaatagtaaaagataacgccctaatgaatgctagttataacttagctttggttgaacagaggttaattctattagcaatcatagaagcgagagaaacaggcaaagggattaatgccaatgatcctttaacagttcatgcaagtagctatatcaatcaatttaacgtagaaaggcatacggcatatcaagccctcaaagatgcttgtaaagacttgtttgcccgtcaattcagttaccaagaaaagcgagaacgaggacgaattaatattacaagtcgatgggtttcgcaaattggctatatggacgatacagcaaccgttgagattatttttgcccctgcggttgttcctctgattacacggctagaggaacagttcacccagtacgatattgagcaaattagcggtttatcgagtgcatatgctgttcgtatgtacgaactgctgatttgttggcgtagcacaggcaaaacaccaattattgagctagacgagtttagaaagcgaataggtgttttagatactgaatacactagaacagataatttaaagatgcgagttattgaattagccctaaaacaaatcaacgaacatacagacatcacagcaagctatgaacaacacaaaaaagggcgagtgattacaggattctcattcaagtttaagcacaagaaacaaaacagcgataaaacgccaaaaaatagcgattctagcccacgtatcgtaaaacatagtcaaatccctccaacattgtaaaacagcctgaaaacgccaaaatgagcgatttagaacatagagcgagccgtgttacaggggaaataatgcgaaatcgtctgtcagatcggtttaaacaaggcgatgaatcagcaatcgacatgatgaaacgtattcaaagtgaaataataaccgatgcaatagcagaccagtgggaaagcaaactggaggagtttggcgtggttttttag

SEQ ID NO: 16 - protein, 327 aa, unidentified
MSDLIVKDNALMNASYNLALVEQRLILLAILEARETGKGINANDPLTVHANSYINQFNVERHTAYQALKDACKDLFARQFSYQEKRERGRINITSRWVSQIGYMDDTATVEVIFAPAVVPLITRLEEQFTQYDIEQISGLSSAYAVRLYELLICWRSTGKTPVIELAEFRKRIGVLDTEYTRTDNLKMRVIELALKQINEHTDITASYEQHKKGRTITGFSFKFKQKKKTELETPKNSDSSPHIEKPSQIPTNIVKQPENAKKDDLGHRASKITGLIMSNGLADRFKRGDESVMNMMKRIKEEITTDATADLWQNKLESMVWFFSHD

SEQ ID NO: 17 - protein, 323 aa, unidentified
MYRWFMSDLIVKDNALMNASYNLDLVEQRLVLLAILEARESGKGINANDPLTVHAESYINQFGVARQTAYQALKGACKDLFARQFSYQEKRERGRANITSRWVSQIAYIDETATVEVIFAPAVVPLITRLEEQFSKYDIEQISSLSSAYAVRLYELLICWRTTGKTPVIDLTEFRKRIGVLDTEYQRMDVFKRGVLELALKQVNEHTDITATYEQHKKGRVITGFSFKFKQKKPKQAEIATETPKTATTDLATTKPLTEPQIAKYSMILCKLGSISDLGNFPDYPTFANWIANILRTPEKADEQIAKRIFTALKTETDYSKKN

SEQ ID NO: 18 - protein, 308 aa, unidentified
MKNGLVVKDNALMNASYNLEVTEQRLILLAIISARETGQGITSDSKLEIHASDYAIQFSVAKETAYEALKSAVNNLFERQFSFREETKKGTGIVRSRWVSRIKYIDDAAILEITFAPDVVPLITRLEEHFTSYQIKQIAQLTSKYAIRLYELLIAWRTTGKVPELELSEFRNRLGIASNEYTAMNNFKSRVLEPSIKQINEHTDITVTYEQHKKGRTITGFSFRFKQKQQAKKIETNRDPNTPDFFIKMTDAQRHLFANKMSEMPEMGKYSQGTESYQQFAIRIADMLLQPEKFRELYPILEKAGFKE

SEQ ID NO: 19 - protein, 318 aa, unidentified
MSELIVKDNALMNASYNLDLVEQRLILLAILEARESGKGINANDPLTVHAESYINQFGVHRTTAYQALKDACKDLFARQFSYQEKRERGRANITSRWVSQIAYIDETGTVEVIFAPAVVPLITRLEEQFTKYDIEQISGLSSAYAVRLYELLICWRTTGKTPIIDLTEFRKRIGVLDTEYQRMDVFKRGVLELALKQVNEHTDITASYEQHKKGRVITGFSFKFKQKKPKQAEIATETPKTATNDPDTTKPLTEPQIAKYSMILCKLGSISDLSNFPDYPAFANWIGNILRNPEKADEQIAKRIFTALKTETDYSKKN

SEQ ID NO: 20 - protein, 322 aa, unidentified
MRLMSELVVKDNALMNASYNLDLVEQRLILLAIVEARESGKGINANDPLTVHAESYINQFGVARQTAYQALKDACDDLFARQFSYQEINERGNTENVRSRWVSEVRYVDAEATVKLIFAPIVIPLITRLEERFTQYEMKQISELSTGYAIRLYELLICWRATGKTPVIELADFRQRMGVLDSEYQRMYDLKKYVLEPSLKQINEHTDITATYEQHKKGRVITGFSFKFKQKKPKQAEIATETPKTATNDQNTIKPLTEPQIAKYSMILCKLGSISDLSNFPDYPSFANWIANILRTPEKADEQAAKRIFTALKTETDYSKKN

SEQ ID NO: 21 - DNA, 33 bp, synthetic construct
  source 1..33: mol_type = other DNA
gcggatccgccatgagcgacctgatcgtgaaag

SEQ ID NO: 22 - DNA, 33 bp, synthetic construct
  source 1..33: mol_type = other DNA
gcggtacctcaaaacacgactccaaactcttcc

SEQ ID NO: 23 - DNA, 112 bp, synthetic construct
  source 1..112: mol_type = other DNA
gtggatccgccatggactacaaagaccatgacggtgattataaagatcatgacatcgattacaaggatgacgatgacaagggagcaagcgacctgatcgtgaaagacaatgc

SEQ ID NO: 24 - DNA, 39 bp, synthetic construct
  source 1..39: mol_type = other DNA
gaggtacctcaaaacacgactcaaactcttccagtttag